European Patent Specification EP 3 807 637 B1, published July 29, 2026. Title: A method of precision cancer therapy. Applicant: King Faisal Specialist Hospital & Research Centre Terramark Markencreation GmbH. The sequence listing filed with the application follows.

SEQUENCE LISTING (11 sequences)

SEQ ID NO: 1 - DNA, 31 bp, Artificial Sequence
  Forward primer
cagcaggatccagaatgctgcaggacttgag

SEQ ID NO: 2 - DNA, 30 bp, Artificial Sequence
  Reverse primer
cgacctctagactattgttcagctccgttt

SEQ ID NO: 3 - DNA, 721 bp, Artificial Sequence
  RPS30M1
ggcaaaactaaggccccaagtaggaatgccttagttttcggggttaacaatgattaacactcctgagcctcacacccacgcgatgccctcagctcctcgctcagcgctctcaccaacagccgtagcccgcagccccgctggacaccgggtctccatccccgcagcgtagcccggaacatggtagctgccatctttacctgctacgccagccttctgtgcgcgcaactgtctggtcccgccccgtcctgcgcgagctgcctgcccaggcaggttcgccggtgcgagcgtaaaggggcggagctaggactgccttgggcggtataaatagcagggaaccgcgcggtcgctcagcagtgacgtgacacgcagcccacggtctgtactgacgcgccctcgcttcttcctctttctcgactccatcttcgcggtagctgggaccgccgttcaggtaagaatggggccttggctgcagccgaagggcttgtagcaggttggctgcggggtcagaaggcgcggggggaaccgaagaacggggcctgctccgtggccctgctccagtccctatccgaactccttgggaggcctggccttccccacgtgagccgccgcgaccaccatcccgtcgcgatcgtttctggaccgctttccactcccaaatctcctttatcccagagcatttcttggcttctcttacaagccgtcttttctttactcagtcgcc

SEQ ID NO: 4 - DNA, 411 bp, Artificial Sequence
  RPS30M-truncated
gatatcggcaaaactaaggccccaagtaggaatgccttagttttcggggttaacaatgattaacactcctgagcctcacacccacgcgatgccctcagctcctcgctcagcgctctcaccaacagccgtagcccgcagccccgctggacaccgggtctccatccccgcagcgtagcccggaacatggtagctgccatctttacctgctacgccagccttctgtgcgcgcaactgtctggtcccgccccgtcctgcgcgagctgcctgcccaggcaggttcgccggtgcgagcgtaaaggggcggagctaggactgccttgggcggtataaatagcagggaaccgcgcggtcgctcagcagtgacgtgacacgcagcccacggtctgtactgacgcgccctcgcttcttcct

SEQ ID NO: 5 - RNA, 11 nt, Artificial Sequence
  AU-rich element
wwwauuuawww

SEQ ID NO: 6 - RNA, 13 nt, Artificial Sequence
  AU-rich element
auuuauuuauuua

SEQ ID NO: 7 - RNA, 17 nt, Artificial Sequence
  AU-rich element
auuuauuuauuuauuua

SEQ ID NO: 8 - RNA, 21 nt, Artificial Sequence
  AU-rich element
auuuauuuauuuauuuauuua

SEQ ID NO: 9 - RNA, 25 nt, Artificial Sequence
  AU-rich element
auuuauuuauuuauuuauuuauuua

SEQ ID NO: 10 - RNA, 12 nt, Artificial Sequence
  AU-rich element repeat unit
  repeat_unit 1..4: /note="1 to 18 repeats"
auuuauuuauuu

SEQ ID NO: 11 - RNA, 20 nt, Artificial Sequence
  AU-rich element
uauuuauuuauuuauuuauu